European Patent Specification EP 3 487 867 B1, published April 1, 2026. Title: METHODS OF PURIFYING FC-CONTAINING PROTEINS. Applicant: AMGEN INC. KAWOOYA, John K. The sequence listing filed with the application follows.

SEQUENCE LISTING (14 sequences)

SEQ ID NO: 1 - protein, 59 aa, Artificial Sequence
  Synthetic polypeptide
ADNKFNKEQQNAFYEILHGPNGNEEQRNAFIQSLKDDPSQSANLLAEAKKLNDAQAPKA

SEQ ID NO: 2 - protein, 59 aa, Artificial Sequence
  Synthetic polypeptide
ADNKFNKEQQNAFYEILHAPNGNEEQRNAFIQSLKDDPSQSANLLAEAKKLNDAQAPKA

SEQ ID NO: 3 - protein, 59 aa, Artificial Sequence
  Synthetic polypeptide
ADNKFNKEQQNAFYEILHLPNGNEEQRNAFIQSLKDDPSQSANLLAEAKKLNDAQAPKA

SEQ ID NO: 4 - protein, 59 aa, Artificial Sequence
  Synthetic polypeptide
ADNKFNKEQQNAFYEILHGPNANEEQRNAFIQSLKDDPSQSANLLAEAKKLNDAQAPKA

SEQ ID NO: 5 - protein, 59 aa, Artificial Sequence
  Synthetic polypeptide
ADNKFNKEQQNAFYEILHGPNLNEEQRNAFIQSLKDDPSQSANLLAEAKKLNDAQAPKA

SEQ ID NO: 6 - protein, 59 aa, Artificial Sequence
  Synthetic polypeptide
ADNKFNKEQQNAFYEILHAPNANEEQRNAFIQSLKDDPSQSANLLAEAKKLNDAQAPKA

SEQ ID NO: 7 - protein, 59 aa, Artificial Sequence
  Synthetic polypeptide
ADNKFNKEQQNAFYEILHLPNGNEEQRNAAIQSLKDDPSQSANLLAEAKKLNDAQAPKA

SEQ ID NO: 8 - protein, 59 aa, Artificial Sequence
  Synthetic polypeptide
ADNKFNKEQQNAFYEILHLPNGNEEQRNAGIQSLKDDPSQSANLLAEAKKLNDAQAPKA

SEQ ID NO: 9 - protein, 59 aa, Artificial Sequence
  Synthetic polypeptide
ADNKFNKEQQNAFYEILHLPNGNEEQRNAFIQSLKDDPSQSANLLAEAKKGNDAQAPKA

SEQ ID NO: 10 - protein, 59 aa, Artificial Sequence
  Synthetic polypeptide
ADNKENKEQQNAFYEILHLPNGNEEGRNAFIQSLKDDPSQSANLLAEAKKLNDAQAPKA

SEQ ID NO: 11 - protein, 59 aa, Artificial Sequence
  Synthetic polypeptide
ADNKFNKEQQNAFYETLHLPNGNEEQGNAFIQSLKDDPSQSANLLAEAKKLNDAQAPKA

SEQ ID NO: 12 - protein, 59 aa, Artificial Sequence
  Synthetic polypeptide
  misc_feature (7)..(7): Xaa can be any naturally occurring amino acid
ADNKFNXEQQNAFYEILHGPNANEEQRNAGIQSLKDDPSQSANLLAEAKKLNDAQAPKA

SEQ ID NO: 13 - protein, 59 aa, Artificial Sequence
  Synthetic polypeptide
ADNKENKEQQNAFYEILHGPNANEEQRNAFIQSLKDDPSQSANLLAEAKKGNDAQAPKA

SEQ ID NO: 14 - protein, 59 aa, Artificial Sequence
  Synthetic polypeptide
ADNKFNKEQQNAFYEILHGPNATEEQRNAFIQSLKDDPSQSANLLAEAKKLNDAQAPKA